European Patent Application EP 4 209 509 A1, published July 12, 2023. Title: ROR1-TARGETED ANTIBODY OR ANTIGEN-BINDING FRAGMENT THEREOF, PREPARATION METHOD AND USE THEREOF. Applicant: Harbour Biomed (Shanghai) Co., Ltd. The sequence listing filed with the application follows.

SEQUENCE LISTING (209 sequences)

SEQ ID NO: 1 - protein, 25 aa, Artificial Sequence
  PR000374 HFWR1 Chothia
EVQLVESGGGLVQPGRSLRLSCTAS

SEQ ID NO: 2 - protein, 25 aa, Artificial Sequence
  PR001352 HFWR1 Chothia, PR001364 HFWR1 Chothia, PR001370 HFWR1 Chothia, PR002572 HFWR1 Chothia, PR002573 HFWR1 Chothia, PR002574 HFWR1 Chothia, PR002575 HFWR1 Chothia, PR002576 HFWR1 Chothia, PR002577
EVQLLESGGGVVQPGRSLRLSCAAS

SEQ ID NO: 3 - protein, 25 aa, Artificial Sequence
  PR001353 HFWR1 Chothia
QVQLVESGGGVVQPGRSLRLSCVAS

SEQ ID NO: 4 - protein, 25 aa, Artificial Sequence
  PR001354 HFWR1 Chothia, PR001357 HFWR1 Chothia, PR001358 HFWR1 Chothia, PR001365 HFWR1 Chothia, PR002562 HFWR1 Chothia, PR002563 HFWR1 Chothia, PR002564 HFWR1 Chothia, PR002565 HFWR1 Chothia, PR002566
QVQLVQSGGGVVQPGRSLRLSCAAS

SEQ ID NO: 5 - protein, 25 aa, Artificial Sequence
  PR001355 HFWR1 Chothia
QVQLVQSGGGLVQPGGSLRLSCAAS

SEQ ID NO: 6 - protein, 25 aa, Artificial Sequence
  PR001356 HFWR1 Chothia, PR001359 HFWR1 Chothia, PR001360 HFWR1 Chothia, PR001363 HFWR1 Chothia, PR001367 HFWR1 Chothia, PR001368 HFWR1 Chothia, PR001369 HFWR1 Chothia, PR001371 HFWR1 Chothia, PR001416
QVQLVESGGGVVQPGRSLRLSCAAS

SEQ ID NO: 7 - protein, 25 aa, Artificial Sequence
  PR001361 HFWR1 Chothia
QVQLVQSGGGVVQPGRSLRLSCTAS

SEQ ID NO: 8 - protein, 25 aa, Artificial Sequence
  PR001362 HFWR1 Chothia
QVQLVESGGGLVQPGGSLRLSCAAS

SEQ ID NO: 9 - protein, 25 aa, Artificial Sequence
  PR001366 HFWR1 Chothia
QVQLVESGGGVVQPGRSLRLSCTAS

SEQ ID NO: 10 - protein, 25 aa, Artificial Sequence
  PR001415 HFWR1 Chothia
EVQLVESGGGVVQPGRSLRLSCAAS

SEQ ID NO: 11 - protein, 7 aa, Artificial Sequence
  PR000374 HCDR1 Chothia
GSDINDY

SEQ ID NO: 12 - protein, 7 aa, Artificial Sequence
  PR001352 HCDR1 Chothia, PR001353 HCDR1 Chothia, PR001354 HCDR1 Chothia, PR001355 HCDR1 Chothia, PR001356 HCDR1 Chothia, PR001357 HCDR1 Chothia, PR001358 HCDR1 Chothia, PR001360 HCDR1 Chothia, PR001365
GFTFSSY

SEQ ID NO: 13 - protein, 7 aa, Artificial Sequence
  PR001359 HCDR1 Chothia, PR001362 HCDR1 Chothia, PR001368 HCDR1 Chothia, PR001416 HCDR1 Chothia
GFTFSTY

SEQ ID NO: 14 - protein, 7 aa, Artificial Sequence
  PR001361 HCDR1 Chothia
GFTFSRY

SEQ ID NO: 15 - protein, 7 aa, Artificial Sequence
  PR001363 HCDR1 Chothia, PR001367 HCDR1 Chothia, PR001417 HCDR1 Chothia
GFSFSSY

SEQ ID NO: 16 - protein, 7 aa, Artificial Sequence
  PR001364 HCDR1 Chothia, PR002572 HCDR1 Chothia, PR002573 HCDR1 Chothia, PR002574 HCDR1 Chothia, PR002575 HCDR1 Chothia, PR002576 HCDR1 Chothia, PR002577 HCDR1 Chothia, PR002578 HCDR1 Chothia, PR002579
GFTFSSF

SEQ ID NO: 17 - protein, 7 aa, Artificial Sequence
  PR001369 HCDR1 Chothia, PR002580 HCDR1 Chothia, PR002581 HCDR1 Chothia, PR002582 HCDR1 Chothia, PR002583 HCDR1 Chothia, PR002584 HCDR1 Chothia, PR002585 HCDR1 Chothia, PR002586 HCDR1 Chothia, PR002587
GFTFSNY

SEQ ID NO: 18 - protein, 7 aa, Artificial Sequence
  PR001415 HCDR1 Chothia
GFTFSNS

SEQ ID NO: 19 - protein, 19 aa, Artificial Sequence
  PR000374 HFWR2 Chothia
PITWVRQAPGQGLEWIGFI

SEQ ID NO: 20 - protein, 19 aa, Artificial Sequence
  PR001352 HFWR2 Chothia, PR001366 HFWR2 Chothia, PR001370 HFWR2 Chothia
GMHWVRQAPGKGLEWVAVK

SEQ ID NO: 21 - protein, 19 aa, Artificial Sequence
  PR001353 HFWR2 Chothia
GMHWVRQAPGKGLEWVSVA

SEQ ID NO: 22 - protein, 19 aa, Artificial Sequence
  PR001354 HFWR2 Chothia, PR001415 HFWR2 Chothia, PR002562 HFWR2 Chothia, PR002563 HFWR2 Chothia, PR002564 HFWR2 Chothia, PR002565 HFWR2 Chothia, PR002566 HFWR2 Chothia, PR002567 HFWR2 Chothia, PR002568
GMHWVRQAPGKGLEWVAIM

SEQ ID NO: 23 - protein, 19 aa, Artificial Sequence
  PR001355 HFWR2 Chothia, PR001357 HFWR2 Chothia, PR001360 HFWR2 Chothia, PR001362 HFWR2 Chothia, PR001364 HFWR2 Chothia, PR001365 HFWR2 Chothia, PR001368 HFWR2 Chothia, PR001416 HFWR2 Chothia, PR001418
GMHWVRQAPGKGLEWVAVI

SEQ ID NO: 24 - protein, 19 aa, Artificial Sequence
  PR001356 HFWR2 Chothia, PR002570 HFWR2 Chothia, PR002571 HFWR2 Chothia
GMHWVRQAPGKGLEWVAVA

SEQ ID NO: 25 - protein, 19 aa, Artificial Sequence
  PR001358 HFWR2 Chothia
AMHWVRQAPGKGLEWVAIM

SEQ ID NO: 26 - protein, 19 aa, Artificial Sequence
  PR001359 HFWR2 Chothia
GMHWVRQAPGKGLEWVAVT

SEQ ID NO: 27 - protein, 19 aa, Artificial Sequence
  PR001361 HFWR2 Chothia, PR001371 HFWR2 Chothia
GMLWVRQAPGKGLEWVAVA

SEQ ID NO: 28 - protein, 19 aa, Artificial Sequence
  PR001363 HFWR2 Chothia, PR001367 HFWR2 Chothia, PR001417 HFWR2 Chothia
AMHWVRQAPGRGLEWVAVI

SEQ ID NO: 29 - protein, 19 aa, Artificial Sequence
  PR001369 HFWR2 Chothia, PR002580 HFWR2 Chothia, PR002581 HFWR2 Chothia, PR002582 HFWR2 Chothia, PR002583 HFWR2 Chothia, PR002584 HFWR2 Chothia, PR002585 HFWR2 Chothia, PR002586 HFWR2 Chothia, PR002587
GIHWVRQAPGKGLEWVAIM

SEQ ID NO: 30 - protein, 19 aa, Artificial Sequence
  PR001419 HFWR2 Chothia
GMHWVRQAPGKGLEWVAII

SEQ ID NO: 31 - protein, 5 aa, Artificial Sequence
  PR000374 HCDR2 Chothia
NSGGS

SEQ ID NO: 32 - protein, 6 aa, Artificial Sequence
  PR001352 HCDR2 Chothia, PR001353 HCDR2 Chothia, PR001366 HCDR2 Chothia, PR001370 HCDR2 Chothia, PR001419 HCDR2 Chothia
WYDGIS

SEQ ID NO: 33 - protein, 6 aa, Artificial Sequence
  PR001354 HCDR2 Chothia, PR001359 HCDR2 Chothia, PR001360 HCDR2 Chothia, PR001362 HCDR2 Chothia, PR001364 HCDR2 Chothia, PR001365 HCDR2 Chothia, PR001368 HCDR2 Chothia, PR001416 HCDR2 Chothia, PR001418
WYDGSD

SEQ ID NO: 34 - protein, 6 aa, Artificial Sequence
  PR001355 HCDR2 Chothia, PR001357 HCDR2 Chothia, PR001358 HCDR2 Chothia, PR001369 HCDR2 Chothia, PR001415 HCDR2 Chothia, PR002580 HCDR2 Chothia, PR002581 HCDR2 Chothia
WYDGSN

SEQ ID NO: 35 - protein, 6 aa, Artificial Sequence
  PR001356 HCDR2 Chothia, PR001361 HCDR2 Chothia, PR001371 HCDR2 Chothia
WYDGVS

SEQ ID NO: 36 - protein, 6 aa, Artificial Sequence
  PR001363 HCDR2 Chothia, PR001367 HCDR2 Chothia, PR001417 HCDR2 Chothia
WYDGGD

SEQ ID NO: 37 - protein, 41 aa, Artificial Sequence
  PR000374 HFWR3 Chothia
TWYASWVKGRFTISRDDSKSIAYLQMNSLKTEDTAVYYCAR

SEQ ID NO: 38 - protein, 41 aa, Artificial Sequence
  PR001352 HFWR3 Chothia, PR001366 HFWR3 Chothia, PR001370 HFWR3 Chothia
QNFADSVKGRFTISRDNSKNTLYLQMNSLRAEDTAVYYCAR

SEQ ID NO: 39 - protein, 41 aa, Artificial Sequence
  PR001353 HFWR3 Chothia
KDYADSVKGRFTISRDNSMNTLFLQMNSLRAEDTAVYYCAR

SEQ ID NO: 40 - protein, 41 aa, Artificial Sequence
  PR001354 HFWR3 Chothia, PR001357 HFWR3 Chothia, PR001359 HFWR3 Chothia, PR001364 HFWR3 Chothia, PR001365 HFWR3 Chothia, PR001415 HFWR3 Chothia, PR001416 HFWR3 Chothia, PR001418 HFWR3 Chothia, PR002562
KDYADSVKGRFTISRDTSKNTLYLQMNSLRAEDTAVYYCAR

SEQ ID NO: 41 - protein, 41 aa, Artificial Sequence
  PR001355 HFWR3 Chothia
KDYADSVKGRFTISRDTSKNTLYLQMNSLRAEDTAVYYCVR

SEQ ID NO: 42 - protein, 41 aa, Artificial Sequence
  PR001356 HFWR3 Chothia, PR002570 HFWR3 Chothia, PR002571 HFWR3 Chothia
EDYADSVKGRFTISRDNAKNTLYLQMNSLRAEDTAVYYCAR

SEQ ID NO: 43 - protein, 41 aa, Artificial Sequence
  PR001358 HFWR3 Chothia, PR001369 HFWR3 Chothia, PR002580 HFWR3 Chothia, PR002581 HFWR3 Chothia, PR002582 HFWR3 Chothia, PR002583 HFWR3 Chothia, PR002584 HFWR3 Chothia, PR002585 HFWR3 Chothia, PR002586
TDYADSVKGRFTISRDTSKNTLFLQMNSLRAEDTAVYYCAR

SEQ ID NO: 44 - protein, 41 aa, Artificial Sequence
  PR001360 HFWR3 Chothia
KDSVDSVKGRFTISRDDSKNTLYLQMNSLRAEDTAVYYCAR

SEQ ID NO: 45 - protein, 41 aa, Artificial Sequence
  PR001361 HFWR3 Chothia, PR001371 HFWR3 Chothia
EDYADSVKGRFTISRDNSMNTLSLQMNSLRAEDTAVYYCAR

SEQ ID NO: 46 - protein, 41 aa, Artificial Sequence
  PR001362 HFWR3 Chothia
EDYADSVKGRFTISRDNSKNTLYLQMNSLRAEDTAVYYCAR

SEQ ID NO: 47 - protein, 41 aa, Artificial Sequence
  PR001363 HFWR3 Chothia
EDSIDSVKGRFTISRDDSKNTLYLQMNSLRAEDTAVYYCAR

SEQ ID NO: 48 - protein, 41 aa, Artificial Sequence
  PR001367 HFWR3 Chothia, PR001417 HFWR3 Chothia
EDYIDSVKGRFTISRDDSKNTLYLQMNSLRAEDTAVYYCAR

SEQ ID NO: 49 - protein, 41 aa, Artificial Sequence
  PR001368 HFWR3 Chothia
TDYADSVKGRFTISRDTSKNTLYLQMNSLRAEDTAVYYCAR

SEQ ID NO: 50 - protein, 41 aa, Artificial Sequence
  PR001419 HFWR3 Chothia
KNYADSVKGRFTISRDMSNNTVYLQMNSLRAEDTAVYYCAK

SEQ ID NO: 51 - protein, 11 aa, Artificial Sequence
  PR000374 HCDR3 Chothia
GYSTYYRDFNI

SEQ ID NO: 52 - protein, 8 aa, Artificial Sequence
  PR001352 HCDR3 Chothia, PR001370 HCDR3 Chothia
DLARSFDL

SEQ ID NO: 53 - protein, 8 aa, Artificial Sequence
  PR001353 HCDR3 Chothia, PR001354 HCDR3 Chothia, PR001355 HCDR3 Chothia, PR001356 HCDR3 Chothia, PR001357 HCDR3 Chothia, PR001358 HCDR3 Chothia, PR001359 HCDR3 Chothia, PR001360 HCDR3 Chothia, PR001361
EQARSFDL

SEQ ID NO: 54 - protein, 8 aa, Artificial Sequence
  PR001362 HCDR3 Chothia
DQARSFDL

SEQ ID NO: 55 - protein, 8 aa, Artificial Sequence
  PR001366 HCDR3 Chothia
DLARSFDI

SEQ ID NO: 56 - protein, 11 aa, Artificial Sequence
  PR000374 HFWR4 Chothia
WGQGTLVTVSS

SEQ ID NO: 57 - protein, 11 aa, Artificial Sequence
  PR001352 HFWR4 Chothia, PR001353 HFWR4 Chothia, PR001354 HFWR4 Chothia, PR001355 HFWR4 Chothia, PR001356 HFWR4 Chothia, PR001357 HFWR4 Chothia, PR001358 HFWR4 Chothia, PR001359 HFWR4 Chothia, PR001360
WGRGTLVTVSS

SEQ ID NO: 58 - protein, 23 aa, Artificial Sequence
  PR000374 LFWR1 Chothia
DIQMTQSPSSLSASVGDRVTINC

SEQ ID NO: 59 - protein, 23 aa, Artificial Sequence
  PR001352 LFWR1 Chothia, PR001371 LFWR1 Chothia
DIQLTQSPSSLSASVGDRVTITC

SEQ ID NO: 60 - protein, 23 aa, Artificial Sequence
  PR001353 LFWR1 Chothia, PR001356 LFWR1 Chothia, PR001358 LFWR1 Chothia, PR001359 LFWR1 Chothia, PR001362 LFWR1 Chothia, PR001364 LFWR1 Chothia, PR001368 LFWR1 Chothia, PR001369 LFWR1 Chothia, PR001370
DIVMTQSPSTLSASVGDRVTITC

SEQ ID NO: 61 - protein, 23 aa, Artificial Sequence
  PR001354 LFWR1 Chothia, PR002562 LFWR1 Chothia, PR002563 LFWR1 Chothia, PR002564 LFWR1 Chothia, PR002565 LFWR1 Chothia, PR002566 LFWR1 Chothia, PR002567 LFWR1 Chothia, PR002568 LFWR1 Chothia, PR002569
DIVMTQSPSSLSASVGDRVTITC

SEQ ID NO: 62 - protein, 23 aa, Artificial Sequence
  PR001355 LFWR1 Chothia
DIQMTQSPSSLSASVGDRVTITC

SEQ ID NO: 63 - protein, 23 aa, Artificial Sequence
  PR001357 LFWR1 Chothia
DIQLTQSPYSLSASVGDRVTITC

SEQ ID NO: 64 - protein, 23 aa, Artificial Sequence
  PR001360 LFWR1 Chothia
DIQMTQSPSTLSASVGDRVTITC

SEQ ID NO: 65 - protein, 23 aa, Artificial Sequence
  PR001361 LFWR1 Chothia, PR001366 LFWR1 Chothia, PR001419 LFWR1 Chothia
DIQLTQSPSTLSASVGDRVTITC

SEQ ID NO: 66 - protein, 23 aa, Artificial Sequence
  PR001363 LFWR1 Chothia, PR001367 LFWR1 Chothia, PR001417 LFWR1 Chothia
DVVMTQSPSTLSASVGDRVTITC

SEQ ID NO: 67 - protein, 23 aa, Artificial Sequence
  PR001365 LFWR1 Chothia
DIQMTQSPYSLSASVGDRVTITC

SEQ ID NO: 68 - protein, 11 aa, Artificial Sequence
  PR000374 LCDR1 Chothia
QASQSIDSNLA

SEQ ID NO: 69 - protein, 11 aa, Artificial Sequence
  PR001352 LCDR1 Chothia, PR001354 LCDR1 Chothia, PR001357 LCDR1 Chothia, PR001360 LCDR1 Chothia, PR001363 LCDR1 Chothia, PR001364 LCDR1 Chothia, PR001365 LCDR1 Chothia, PR001367 LCDR1 Chothia, PR001369
RASQTINNWLA

SEQ ID NO: 70 - protein, 11 aa, Artificial Sequence
  PR001353 LCDR1 Chothia, PR001419 LCDR1 Chothia
RASQSISSWLA

SEQ ID NO: 71 - protein, 11 aa, Artificial Sequence
  PR001355 LCDR1 Chothia
RASQTMNNWLA

SEQ ID NO: 72 - protein, 11 aa, Artificial Sequence
  PR001356 LCDR1 Chothia, PR001370 LCDR1 Chothia, PR002570 LCDR1 Chothia, PR002571 LCDR1 Chothia
RASQSINNWLA

SEQ ID NO: 73 - protein, 11 aa, Artificial Sequence
  PR001358 LCDR1 Chothia, PR001361 LCDR1 Chothia, PR001362 LCDR1 Chothia, PR001366 LCDR1 Chothia, PR001368 LCDR1 Chothia, PR001417 LCDR1 Chothia
RASQSINSWLA

SEQ ID NO: 74 - protein, 11 aa, Artificial Sequence
  PR001359 LCDR1 Chothia
RASQSVNNWLA

SEQ ID NO: 75 - protein, 15 aa, Artificial Sequence
  PR000374 LFWR2 Chothia
WFQQKPGQPPKLLIY

SEQ ID NO: 76 - protein, 15 aa, Artificial Sequence
  PR001352 LFWR2 Chothia, PR001353 LFWR2 Chothia, PR001354 LFWR2 Chothia, PR001355 LFWR2 Chothia, PR001356 LFWR2 Chothia, PR001357 LFWR2 Chothia, PR001358 LFWR2 Chothia, PR001359 LFWR2 Chothia, PR001360
WYQQKPGKAPKLLIY

SEQ ID NO: 77 - protein, 7 aa, Artificial Sequence
  PR000374 LCDR2 Chothia
RASNLAS

SEQ ID NO: 78 - protein, 7 aa, Artificial Sequence
  PR001352 LCDR2 Chothia, PR001353 LCDR2 Chothia, PR001354 LCDR2 Chothia, PR001355 LCDR2 Chothia, PR001356 LCDR2 Chothia, PR001357 LCDR2 Chothia, PR001359 LCDR2 Chothia, PR001360 LCDR2 Chothia, PR001361
KASSLES

SEQ ID NO: 79 - protein, 7 aa, Artificial Sequence
  PR001358 LCDR2 Chothia
KASNLES

SEQ ID NO: 80 - protein, 32 aa, Artificial Sequence
  PR000374 LFWR3 Chothia
GVPDRFSGSGSGTDFTLTISSLEAEDVATYYC

SEQ ID NO: 81 - protein, 32 aa, Artificial Sequence
  PR001352 LFWR3 Chothia, PR001353 LFWR3 Chothia, PR001354 LFWR3 Chothia, PR001356 LFWR3 Chothia, PR001357 LFWR3 Chothia, PR001358 LFWR3 Chothia, PR001359 LFWR3 Chothia, PR001360 LFWR3 Chothia, PR001361
GVPSRFSGSGSGTEFTLTISSLQPDDFATYYC

SEQ ID NO: 82 - protein, 32 aa, Artificial Sequence
  PR001355 LFWR3 Chothia
GVPSRFSGSGSGTEFTLTISSLQPDDSATYYC

SEQ ID NO: 83 - protein, 12 aa, Artificial Sequence
  PR000374 LCDR3 Chothia
LGGVGAVSYRTS

SEQ ID NO: 84 - protein, 11 aa, Artificial Sequence
  PR001352 LCDR3 Chothia, PR001354 LCDR3 Chothia, PR001355 LCDR3 Chothia, PR001363 LCDR3 Chothia, PR001364 LCDR3 Chothia, PR001367 LCDR3 Chothia, PR001369 LCDR3 Chothia, PR001370 LCDR3 Chothia, PR001371
QQYNSYSPMYT

SEQ ID NO: 85 - protein, 11 aa, Artificial Sequence
  PR001353 LCDR3 Chothia, PR001356 LCDR3 Chothia, PR001358 LCDR3 Chothia, PR001359 LCDR3 Chothia, PR001361 LCDR3 Chothia, PR001362 LCDR3 Chothia, PR001366 LCDR3 Chothia, PR001368 LCDR3 Chothia, PR002570
QQYKSYSPMYT

SEQ ID NO: 86 - protein, 11 aa, Artificial Sequence
  PR001357 LCDR3 Chothia, PR001365 LCDR3 Chothia
QQYKLYSPMYT

SEQ ID NO: 87 - protein, 11 aa, Artificial Sequence
  PR001360 LCDR3 Chothia
QQYNIYSPMYT

SEQ ID NO: 88 - protein, 10 aa, Artificial Sequence
  PR000374 LFWR4 Chothia
FGGGTKVEIK

SEQ ID NO: 89 - protein, 10 aa, Artificial Sequence
  PR001352 LFWR4 Chothia, PR001353 LFWR4 Chothia, PR001354 LFWR4 Chothia, PR001356 LFWR4 Chothia, PR001357 LFWR4 Chothia, PR001359 LFWR4 Chothia, PR001360 LFWR4 Chothia, PR001362 LFWR4 Chothia, PR001363
FGQGTKVEIK

SEQ ID NO: 90 - protein, 10 aa, Artificial Sequence
  PR001355 LFWR4 Chothia, PR001418 LFWR4 Chothia
FGQGTKLEIK

SEQ ID NO: 91 - protein, 10 aa, Artificial Sequence
  PR001358 LFWR4 Chothia, PR001361 LFWR4 Chothia, PR001366 LFWR4 Chothia, PR001370 LFWR4 Chothia
FGQGTKVDIK

SEQ ID NO: 92 - protein, 119 aa, Artificial Sequence
  PR000374 VH
EVQLVESGGGLVQPGRSLRLSCTASGSDINDYPITWVRQAPGQGLEWIGFINSGGSTWYASWVKGRFTISRDDSKSIAYLQMNSLKTEDTAVYYCARGYSTYYRDFNIWGQGTLVTVSS

SEQ ID NO: 93 - protein, 117 aa, Artificial Sequence
  PR001352 VH, PR001370 VH
EVQLLESGGGVVQPGRSLRLSCAASGFTFSSYGMHWVRQAPGKGLEWVAVKWYDGISQNFADSVKGRFTISRDNSKNTLYLQMNSLRAEDTAVYYCARDLARSFDLWGRGTLVTVSS

SEQ ID NO: 94 - protein, 117 aa, Artificial Sequence
  PR001353 VH
QVQLVESGGGVVQPGRSLRLSCVASGFTFSSYGMHWVRQAPGKGLEWVSVAWYDGISKDYADSVKGRFTISRDNSMNTLFLQMNSLRAEDTAVYYCAREQARSFDLWGRGTLVTVSS

SEQ ID NO: 95 - protein, 117 aa, Artificial Sequence
  PR001354 VH, PR002562 VH, PR002563 VH
QVQLVQSGGGVVQPGRSLRLSCAASGFTFSSYGMHWVRQAPGKGLEWVAIMWYDGSDKDYADSVKGRFTISRDTSKNTLYLQMNSLRAEDTAVYYCAREQARSFDLWGRGTLVTVSS

SEQ ID NO: 96 - protein, 117 aa, Artificial Sequence
  PR001355 VH
QVQLVQSGGGLVQPGGSLRLSCAASGFTFSSYGMHWVRQAPGKGLEWVAVIWYDGSNKDYADSVKGRFTISRDTSKNTLYLQMNSLRAEDTAVYYCVREQARSFDLWGRGTLVTVSS

SEQ ID NO: 97 - protein, 117 aa, Artificial Sequence
  PR001356 VH
QVQLVESGGGVVQPGRSLRLSCAASGFTFSSYGMHWVRQAPGKGLEWVAVAWYDGVSEDYADSVKGRFTISRDNAKNTLYLQMNSLRAEDTAVYYCAREQARSFDLWGRGTLVTVSS

SEQ ID NO: 98 - protein, 117 aa, Artificial Sequence
  PR001357 VH
QVQLVQSGGGVVQPGRSLRLSCAASGFTFSSYGMHWVRQAPGKGLEWVAVIWYDGSNKDYADSVKGRFTISRDTSKNTLYLQMNSLRAEDTAVYYCAREQARSFDLWGRGTLVTVSS

SEQ ID NO: 99 - protein, 117 aa, Artificial Sequence
  PR001358 VH
QVQLVQSGGGVVQPGRSLRLSCAASGFTFSSYAMHWVRQAPGKGLEWVAIMWYDGSNTDYADSVKGRFTISRDTSKNTLFLQMNSLRAEDTAVYYCAREQARSFDLWGRGTLVTVSS

SEQ ID NO: 100 - protein, 117 aa, Artificial Sequence
  PR001359 VH
QVQLVESGGGVVQPGRSLRLSCAASGFTFSTYGMHWVRQAPGKGLEWVAVTWYDGSDKDYADSVKGRFTISRDTSKNTLYLQMNSLRAEDTAVYYCAREQARSFDLWGRGTLVTVSS

SEQ ID NO: 101 - protein, 117 aa, Artificial Sequence
  PR001360 VH
QVQLVESGGGVVQPGRSLRLSCAASGFTFSSYGMHWVRQAPGKGLEWVAVIWYDGSDKDSVDSVKGRFTISRDDSKNTLYLQMNSLRAEDTAVYYCAREQARSFDLWGRGTLVTVSS

SEQ ID NO: 102 - protein, 117 aa, Artificial Sequence
  PR001361 VH
QVQLVQSGGGVVQPGRSLRLSCTASGFTFSRYGMLWVRQAPGKGLEWVAVAWYDGVSEDYADSVKGRFTISRDNSMNTLSLQMNSLRAEDTAVYYCAREQARSFDLWGRGTLVTVSS

SEQ ID NO: 103 - protein, 117 aa, Artificial Sequence
  PR001362 VH
QVQLVESGGGLVQPGGSLRLSCAASGFTFSTYGMHWVRQAPGKGLEWVAVIWYDGSDEDYADSVKGRFTISRDNSKNTLYLQMNSLRAEDTAVYYCARDQARSFDLWGRGTLVTVSS

SEQ ID NO: 104 - protein, 117 aa, Artificial Sequence
  PR001363 VH
QVQLVESGGGVVQPGRSLRLSCAASGFSFSSYAMHWVRQAPGRGLEWVAVIWYDGGDEDSIDSVKGRFTISRDDSKNTLYLQMNSLRAEDTAVYYCAREQARSFDLWGRGTLVTVSS

SEQ ID NO: 105 - protein, 117 aa, Artificial Sequence
  PR001364 VH, PR002572 VH, PR002573 VH
EVQLLESGGGVVQPGRSLRLSCAASGFTFSSFGMHWVRQAPGKGLEWVAVIWYDGSDKDYADSVKGRFTISRDTSKNTLYLQMNSLRAEDTAVYYCAREQARSFDLWGRGTLVTVSS

SEQ ID NO: 106 - protein, 117 aa, Artificial Sequence
  PR001365 VH
QVQLVQSGGGVVQPGRSLRLSCAASGFTFSSYGMHWVRQAPGKGLEWVAVIWYDGSDKDYADSVKGRFTISRDTSKNTLYLQMNSLRAEDTAVYYCAREQARSFDLWGRGTLVTVSS

SEQ ID NO: 107 - protein, 117 aa, Artificial Sequence
  PR001366 VH
QVQLVESGGGVVQPGRSLRLSCTASGFTFSSYGMHWVRQAPGKGLEWVAVKWYDGISQNFADSVKGRFTISRDNSKNTLYLQMNSLRAEDTAVYYCARDLARSFDIWGRGTLVTVSS

SEQ ID NO: 108 - protein, 117 aa, Artificial Sequence
  PR001367 VH, PR001417 VH
QVQLVESGGGVVQPGRSLRLSCAASGFSFSSYAMHWVRQAPGRGLEWVAVIWYDGGDEDYIDSVKGRFTISRDDSKNTLYLQMNSLRAEDTAVYYCAREQARSFDLWGRGTLVTVSS

SEQ ID NO: 109 - protein, 117 aa, Artificial Sequence
  PR001368 VH
QVQLVESGGGVVQPGRSLRLSCAASGFTFSTYGMHWVRQAPGKGLEWVAVIWYDGSDTDYADSVKGRFTISRDTSKNTLYLQMNSLRAEDTAVYYCAREQARSFDLWGRGTLVTVSS

SEQ ID NO: 110 - protein, 117 aa, Artificial Sequence
  PR001369 VH, PR002580 VH, PR002581 VH
QVQLVESGGGVVQPGRSLRLSCAASGFTFSNYGIHWVRQAPGKGLEWVAIMWYDGSNTDYADSVKGRFTISRDTSKNTLFLQMNSLRAEDTAVYYCAREQARSFDLWGRGTLVTVSS

SEQ ID NO: 111 - protein, 117 aa, Artificial Sequence
  PR001371 VH
QVQLVESGGGVVQPGRSLRLSCAASGFTFSSYGMLWVRQAPGKGLEWVAVAWYDGVSEDYADSVKGRFTISRDNSMNTLSLQMNSLRAEDTAVYYCAREQARSFDLWGRGTLVTVSS

SEQ ID NO: 112 - protein, 117 aa, Artificial Sequence
  PR001415 VH
EVQLVESGGGVVQPGRSLRLSCAASGFTFSNSGMHWVRQAPGKGLEWVAIMWYDGSNKDYADSVKGRFTISRDTSKNTLYLQMNSLRAEDTAVYYCAREQARSFDLWGRGTLVTVSS

SEQ ID NO: 113 - protein, 117 aa, Artificial Sequence
  PR001416 VH
QVQLVESGGGVVQPGRSLRLSCAASGFTFSTYGMHWVRQAPGKGLEWVAVIWYDGSDKDYADSVKGRFTISRDTSKNTLYLQMNSLRAEDTAVYYCAREQARSFDLWGRGTLVTVSS

SEQ ID NO: 114 - protein, 117 aa, Artificial Sequence
  PR001418 VH
QVQLVESGGGVVQPGRSLRLSCAASGFTFSSYGMHWVRQAPGKGLEWVAVIWYDGSDKDYADSVKGRFTISRDTSKNTLYLQMNSLRAEDTAVYYCAREQARSFDLWGRGTLVTVSS

SEQ ID NO: 115 - protein, 117 aa, Artificial Sequence
  PR001419 VH
QVQLVESGGGVVQPGRSLRLSCAASGFTFSSYGMHWVRQAPGKGLEWVAIIWYDGISKNYADSVKGRFTISRDMSNNTVYLQMNSLRAEDTAVYYCAKEQARSFDLWGRGTLVTVSS

SEQ ID NO: 116 - protein, 110 aa, Artificial Sequence
  PR000374 VL
DIQMTQSPSSLSASVGDRVTINCQASQSIDSNLAWFQQKPGQPPKLLIYRASNLASGVPDRFSGSGSGTDFTLTISSLEAEDVATYYCLGGVGAVSYRTSFGGGTKVEIK

SEQ ID NO: 117 - protein, 109 aa, Artificial Sequence
  PR001352 VL, PR001371 VL
DIQLTQSPSSLSASVGDRVTITCRASQTINNWLAWYQQKPGKAPKLLIYKASSLESGVPSRFSGSGSGTEFTLTISSLQPDDFATYYCQQYNSYSPMYTFGQGTKVEIK

SEQ ID NO: 118 - protein, 109 aa, Artificial Sequence
  PR001353 VL
DIVMTQSPSTLSASVGDRVTITCRASQSISSWLAWYQQKPGKAPKLLIYKASSLESGVPSRFSGSGSGTEFTLTISSLQPDDFATYYCQQYKSYSPMYTFGQGTKVEIK

SEQ ID NO: 119 - protein, 109 aa, Artificial Sequence
  PR001354 VL, PR002564 VL, PR002567 VL
DIVMTQSPSSLSASVGDRVTITCRASQTINNWLAWYQQKPGKAPKLLIYKASSLESGVPSRFSGSGSGTEFTLTISSLQPDDFATYYCQQYNSYSPMYTFGQGTKVEIK

SEQ ID NO: 120 - protein, 109 aa, Artificial Sequence
  PR001355 VL
DIQMTQSPSSLSASVGDRVTITCRASQTMNNWLAWYQQKPGKAPKLLIYKASSLESGVPSRFSGSGSGTEFTLTISSLQPDDSATYYCQQYNSYSPMYTFGQGTKLEIK

SEQ ID NO: 121 - protein, 109 aa, Artificial Sequence
  PR001356 VL, PR002570 VL, PR002571 VL
DIVMTQSPSTLSASVGDRVTITCRASQSINNWLAWYQQKPGKAPKLLIYKASSLESGVPSRFSGSGSGTEFTLTISSLQPDDFATYYCQQYKSYSPMYTFGQGTKVEIK

SEQ ID NO: 122 - protein, 109 aa, Artificial Sequence
  PR001357 VL
DIQLTQSPYSLSASVGDRVTITCRASQTINNWLAWYQQKPGKAPKLLIYKASSLESGVPSRFSGSGSGTEFTLTISSLQPDDFATYYCQQYKLYSPMYTFGQGTKVEIK

SEQ ID NO: 123 - protein, 109 aa, Artificial Sequence
  PR001358 VL
DIVMTQSPSTLSASVGDRVTITCRASQSINSWLAWYQQKPGKAPKLLIYKASNLESGVPSRFSGSGSGTEFTLTISSLQPDDFATYYCQQYKSYSPMYTFGQGTKVDIK

SEQ ID NO: 124 - protein, 109 aa, Artificial Sequence
  PR001359 VL
DIVMTQSPSTLSASVGDRVTITCRASQSVNNWLAWYQQKPGKAPKLLIYKASSLESGVPSRFSGSGSGTEFTLTISSLQPDDFATYYCQQYKSYSPMYTFGQGTKVEIK

SEQ ID NO: 125 - protein, 109 aa, Artificial Sequence
  PR001360 VL
DIQMTQSPSTLSASVGDRVTITCRASQTINNWLAWYQQKPGKAPKLLIYKASSLESGVPSRFSGSGSGTEFTLTISSLQPDDFATYYCQQYNIYSPMYTFGQGTKVEIK

SEQ ID NO: 126 - protein, 109 aa, Artificial Sequence
  PR001361 VL, PR001366 VL
DIQLTQSPSTLSASVGDRVTITCRASQSINSWLAWYQQKPGKAPKLLIYKASSLESGVPSRFSGSGSGTEFTLTISSLQPDDFATYYCQQYKSYSPMYTFGQGTKVDIK

SEQ ID NO: 127 - protein, 109 aa, Artificial Sequence
  PR001362 VL, PR001368 VL
DIVMTQSPSTLSASVGDRVTITCRASQSINSWLAWYQQKPGKAPKLLIYKASSLESGVPSRFSGSGSGTEFTLTISSLQPDDFATYYCQQYKSYSPMYTFGQGTKVEIK

SEQ ID NO: 128 - protein, 109 aa, Artificial Sequence
  PR001363 VL, PR001367 VL
DVVMTQSPSTLSASVGDRVTITCRASQTINNWLAWYQQKPGKAPKLLIYKASSLESGVPSRFSGSGSGTEFTLTISSLQPDDFATYYCQQYNSYSPMYTFGQGTKVEIK

SEQ ID NO: 129 - protein, 109 aa, Artificial Sequence
  PR001364 VL, PR001369 VL, PR001415 VL, PR001416 VL, PR002574 VL, PR002577 VL, PR002582 VL, PR002585 VL
DIVMTQSPSTLSASVGDRVTITCRASQTINNWLAWYQQKPGKAPKLLIYKASSLESGVPSRFSGSGSGTEFTLTISSLQPDDFATYYCQQYNSYSPMYTFGQGTKVEIK

SEQ ID NO: 130 - protein, 109 aa, Artificial Sequence
  PR001365 VL
DIQMTQSPYSLSASVGDRVTITCRASQTINNWLAWYQQKPGKAPKLLIYKASSLESGVPSRFSGSGSGTEFTLTISSLQPDDFATYYCQQYKLYSPMYTFGQGTKVEIK

SEQ ID NO: 131 - protein, 109 aa, Artificial Sequence
  PR001370 VL
DIVMTQSPSTLSASVGDRVTITCRASQSINNWLAWYQQKPGKAPKLLIYKASSLESGVPSRFSGSGSGTEFTLTISSLQPDDFATYYCQQYNSYSPMYTFGQGTKVDIK

SEQ ID NO: 132 - protein, 109 aa, Artificial Sequence
  PR001417 VL
DVVMTQSPSTLSASVGDRVTITCRASQSINSWLAWYQQKPGKAPKLLIYKASSLESGVPSRFSGSGSGTEFTLTISSLQPDDFATYYCQQYNSYSPMYTFGQGTKVEIK

SEQ ID NO: 133 - protein, 109 aa, Artificial Sequence
  PR001418 VL
DIVMTQSPSTLSASVGDRVTITCRASQTINNWLAWYQQKPGKAPKLLIYKASSLESGVPSRFSGSGSGTEFTLTISSLQPDDFATYYCQQYNSYSPMYTFGQGTKLEIK

SEQ ID NO: 134 - protein, 109 aa, Artificial Sequence
  PR001419 VL
DIQLTQSPSTLSASVGDRVTITCRASQSISSWLAWYQQKPGKAPKLLIYKASSLESGVPSRFSGSGSGTEFTLTISSLQPDDFATYYCQQYNSYSPMYTFGQGTKVEIK

SEQ ID NO: 135 - protein, 449 aa, Artificial Sequence
  PR000374 HC
EVQLVESGGGLVQPGRSLRLSCTASGSDINDYPITWVRQAPGQGLEWIGFINSGGSTWYASWVKGRFTISRDDSKSIAYLQMNSLKTEDTAVYYCARGYSTYYRDFNIWGQGTLVTVSSASTKGPSVFPLAPSSKSTSGGTAALGCLVKDYFPEPVTVSWNSGALTSGVHTFPAVLQSSGLYSLSSVVTVPSSSLGTQTYICNVNHKPSNTKVDKKVEPKSCDKTHTCPPCPAPELLGGPSVFLFPPKPKDTLMISRTPEVTCVVVDVSHEDPEVKFNWYVDGVEVHNAKTKPREEQYNSTYRVVSVLTVLHQDWLNGKEYKCKVSNKALPAPIEKTISKAKGQPREPQVYTLPPSREEMTKNQVSLTCLVKGFYPSDIAVEWESNGQPENNYKTTPPVLDSDGSFFLYSKLTVDKSRWQQGNVFSCSVMHEALHNHYTQKSLSLSPGK

SEQ ID NO: 136 - protein, 447 aa, Artificial Sequence
  PR001352 HC, PR001370 HC
EVQLLESGGGVVQPGRSLRLSCAASGFTFSSYGMHWVRQAPGKGLEWVAVKWYDGISQNFADSVKGRFTISRDNSKNTLYLQMNSLRAEDTAVYYCARDLARSFDLWGRGTLVTVSSASTKGPSVFPLAPSSKSTSGGTAALGCLVKDYFPEPVTVSWNSGALTSGVHTFPAVLQSSGLYSLSSVVTVPSSSLGTQTYICNVNHKPSNTKVDKKVEPKSCDKTHTCPPCPAPELLGGPSVFLFPPKPKDTLMISRTPEVTCVVVDVSHEDPEVKFNWYVDGVEVHNAKTKPREEQYNSTYRVVSVLTVLHQDWLNGKEYKCKVSNKALPAPIEKTISKAKGQPREPQVYTLPPSREEMTKNQVSLTCLVKGFYPSDIAVEWESNGQPENNYKTTPPVLDSDGSFFLYSKLTVDKSRWQQGNVFSCSVMHEALHNHYTQKSLSLSPGK

SEQ ID NO: 137 - protein, 447 aa, Artificial Sequence
  PR001353 HC
QVQLVESGGGVVQPGRSLRLSCVASGFTFSSYGMHWVRQAPGKGLEWVSVAWYDGISKDYADSVKGRFTISRDNSMNTLFLQMNSLRAEDTAVYYCAREQARSFDLWGRGTLVTVSSASTKGPSVFPLAPSSKSTSGGTAALGCLVKDYFPEPVTVSWNSGALTSGVHTFPAVLQSSGLYSLSSVVTVPSSSLGTQTYICNVNHKPSNTKVDKKVEPKSCDKTHTCPPCPAPELLGGPSVFLFPPKPKDTLMISRTPEVTCVVVDVSHEDPEVKFNWYVDGVEVHNAKTKPREEQYNSTYRVVSVLTVLHQDWLNGKEYKCKVSNKALPAPIEKTISKAKGQPREPQVYTLPPSREEMTKNQVSLTCLVKGFYPSDIAVEWESNGQPENNYKTTPPVLDSDGSFFLYSKLTVDKSRWQQGNVFSCSVMHEALHNHYTQKSLSLSPGK

SEQ ID NO: 138 - protein, 447 aa, Artificial Sequence
  PR001354 HC, PR002562 HC, PR002563 HC
QVQLVQSGGGVVQPGRSLRLSCAASGFTFSSYGMHWVRQAPGKGLEWVAIMWYDGSDKDYADSVKGRFTISRDTSKNTLYLQMNSLRAEDTAVYYCAREQARSFDLWGRGTLVTVSSASTKGPSVFPLAPSSKSTSGGTAALGCLVKDYFPEPVTVSWNSGALTSGVHTFPAVLQSSGLYSLSSVVTVPSSSLGTQTYICNVNHKPSNTKVDKKVEPKSCDKTHTCPPCPAPELLGGPSVFLFPPKPKDTLMISRTPEVTCVVVDVSHEDPEVKFNWYVDGVEVHNAKTKPREEQYNSTYRVVSVLTVLHQDWLNGKEYKCKVSNKALPAPIEKTISKAKGQPREPQVYTLPPSREEMTKNQVSLTCLVKGFYPSDIAVEWESNGQPENNYKTTPPVLDSDGSFFLYSKLTVDKSRWQQGNVFSCSVMHEALHNHYTQKSLSLSPGK

SEQ ID NO: 139 - protein, 447 aa, Artificial Sequence
  PR001355 HC
QVQLVQSGGGLVQPGGSLRLSCAASGFTFSSYGMHWVRQAPGKGLEWVAVIWYDGSNKDYADSVKGRFTISRDTSKNTLYLQMNSLRAEDTAVYYCVREQARSFDLWGRGTLVTVSSASTKGPSVFPLAPSSKSTSGGTAALGCLVKDYFPEPVTVSWNSGALTSGVHTFPAVLQSSGLYSLSSVVTVPSSSLGTQTYICNVNHKPSNTKVDKKVEPKSCDKTHTCPPCPAPELLGGPSVFLFPPKPKDTLMISRTPEVTCVVVDVSHEDPEVKFNWYVDGVEVHNAKTKPREEQYNSTYRVVSVLTVLHQDWLNGKEYKCKVSNKALPAPIEKTISKAKGQPREPQVYTLPPSREEMTKNQVSLTCLVKGFYPSDIAVEWESNGQPENNYKTTPPVLDSDGSFFLYSKLTVDKSRWQQGNVFSCSVMHEALHNHYTQKSLSLSPGK

SEQ ID NO: 140 - protein, 447 aa, Artificial Sequence
  PR001356 HC
QVQLVESGGGVVQPGRSLRLSCAASGFTFSSYGMHWVRQAPGKGLEWVAVAWYDGVSEDYADSVKGRFTISRDNAKNTLYLQMNSLRAEDTAVYYCAREQARSFDLWGRGTLVTVSSASTKGPSVFPLAPSSKSTSGGTAALGCLVKDYFPEPVTVSWNSGALTSGVHTFPAVLQSSGLYSLSSVVTVPSSSLGTQTYICNVNHKPSNTKVDKKVEPKSCDKTHTCPPCPAPELLGGPSVFLFPPKPKDTLMISRTPEVTCVVVDVSHEDPEVKFNWYVDGVEVHNAKTKPREEQYNSTYRVVSVLTVLHQDWLNGKEYKCKVSNKALPAPIEKTISKAKGQPREPQVYTLPPSREEMTKNQVSLTCLVKGFYPSDIAVEWESNGQPENNYKTTPPVLDSDGSFFLYSKLTVDKSRWQQGNVFSCSVMHEALHNHYTQKSLSLSPGK

SEQ ID NO: 141 - protein, 447 aa, Artificial Sequence
  PR001357 HC
QVQLVQSGGGVVQPGRSLRLSCAASGFTFSSYGMHWVRQAPGKGLEWVAVIWYDGSNKDYADSVKGRFTISRDTSKNTLYLQMNSLRAEDTAVYYCAREQARSFDLWGRGTLVTVSSASTKGPSVFPLAPSSKSTSGGTAALGCLVKDYFPEPVTVSWNSGALTSGVHTFPAVLQSSGLYSLSSVVTVPSSSLGTQTYICNVNHKPSNTKVDKKVEPKSCDKTHTCPPCPAPELLGGPSVFLFPPKPKDTLMISRTPEVTCVVVDVSHEDPEVKFNWYVDGVEVHNAKTKPREEQYNSTYRVVSVLTVLHQDWLNGKEYKCKVSNKALPAPIEKTISKAKGQPREPQVYTLPPSREEMTKNQVSLTCLVKGFYPSDIAVEWESNGQPENNYKTTPPVLDSDGSFFLYSKLTVDKSRWQQGNVFSCSVMHEALHNHYTQKSLSLSPGK

SEQ ID NO: 142 - protein, 447 aa, Artificial Sequence
  PR001358 HC
QVQLVQSGGGVVQPGRSLRLSCAASGFTFSSYAMHWVRQAPGKGLEWVAIMWYDGSNTDYADSVKGRFTISRDTSKNTLFLQMNSLRAEDTAVYYCAREQARSFDLWGRGTLVTVSSASTKGPSVFPLAPSSKSTSGGTAALGCLVKDYFPEPVTVSWNSGALTSGVHTFPAVLQSSGLYSLSSVVTVPSSSLGTQTYICNVNHKPSNTKVDKKVEPKSCDKTHTCPPCPAPELLGGPSVFLFPPKPKDTLMISRTPEVTCVVVDVSHEDPEVKFNWYVDGVEVHNAKTKPREEQYNSTYRVVSVLTVLHQDWLNGKEYKCKVSNKALPAPIEKTISKAKGQPREPQVYTLPPSREEMTKNQVSLTCLVKGFYPSDIAVEWESNGQPENNYKTTPPVLDSDGSFFLYSKLTVDKSRWQQGNVFSCSVMHEALHNHYTQKSLSLSPGK

SEQ ID NO: 143 - protein, 447 aa, Artificial Sequence
  PR001359 HC
QVQLVESGGGVVQPGRSLRLSCAASGFTFSTYGMHWVRQAPGKGLEWVAVTWYDGSDKDYADSVKGRFTISRDTSKNTLYLQMNSLRAEDTAVYYCAREQARSFDLWGRGTLVTVSSASTKGPSVFPLAPSSKSTSGGTAALGCLVKDYFPEPVTVSWNSGALTSGVHTFPAVLQSSGLYSLSSVVTVPSSSLGTQTYICNVNHKPSNTKVDKKVEPKSCDKTHTCPPCPAPELLGGPSVFLFPPKPKDTLMISRTPEVTCVVVDVSHEDPEVKFNWYVDGVEVHNAKTKPREEQYNSTYRVVSVLTVLHQDWLNGKEYKCKVSNKALPAPIEKTISKAKGQPREPQVYTLPPSREEMTKNQVSLTCLVKGFYPSDIAVEWESNGQPENNYKTTPPVLDSDGSFFLYSKLTVDKSRWQQGNVFSCSVMHEALHNHYTQKSLSLSPGK

SEQ ID NO: 144 - protein, 447 aa, Artificial Sequence
  PR001360 HC
QVQLVESGGGVVQPGRSLRLSCAASGFTFSSYGMHWVRQAPGKGLEWVAVIWYDGSDKDSVDSVKGRFTISRDDSKNTLYLQMNSLRAEDTAVYYCAREQARSFDLWGRGTLVTVSSASTKGPSVFPLAPSSKSTSGGTAALGCLVKDYFPEPVTVSWNSGALTSGVHTFPAVLQSSGLYSLSSVVTVPSSSLGTQTYICNVNHKPSNTKVDKKVEPKSCDKTHTCPPCPAPELLGGPSVFLFPPKPKDTLMISRTPEVTCVVVDVSHEDPEVKFNWYVDGVEVHNAKTKPREEQYNSTYRVVSVLTVLHQDWLNGKEYKCKVSNKALPAPIEKTISKAKGQPREPQVYTLPPSREEMTKNQVSLTCLVKGFYPSDIAVEWESNGQPENNYKTTPPVLDSDGSFFLYSKLTVDKSRWQQGNVFSCSVMHEALHNHYTQKSLSLSPGK

SEQ ID NO: 145 - protein, 447 aa, Artificial Sequence
  PR001361 HC
QVQLVQSGGGVVQPGRSLRLSCTASGFTFSRYGMLWVRQAPGKGLEWVAVAWYDGVSEDYADSVKGRFTISRDNSMNTLSLQMNSLRAEDTAVYYCAREQARSFDLWGRGTLVTVSSASTKGPSVFPLAPSSKSTSGGTAALGCLVKDYFPEPVTVSWNSGALTSGVHTFPAVLQSSGLYSLSSVVTVPSSSLGTQTYICNVNHKPSNTKVDKKVEPKSCDKTHTCPPCPAPELLGGPSVFLFPPKPKDTLMISRTPEVTCVVVDVSHEDPEVKFNWYVDGVEVHNAKTKPREEQYNSTYRVVSVLTVLHQDWLNGKEYKCKVSNKALPAPIEKTISKAKGQPREPQVYTLPPSREEMTKNQVSLTCLVKGFYPSDIAVEWESNGQPENNYKTTPPVLDSDGSFFLYSKLTVDKSRWQQGNVFSCSVMHEALHNHYTQKSLSLSPGK

SEQ ID NO: 146 - protein, 447 aa, Artificial Sequence
  PR001362 HC
QVQLVESGGGLVQPGGSLRLSCAASGFTFSTYGMHWVRQAPGKGLEWVAVIWYDGSDEDYADSVKGRFTISRDNSKNTLYLQMNSLRAEDTAVYYCARDQARSFDLWGRGTLVTVSSASTKGPSVFPLAPSSKSTSGGTAALGCLVKDYFPEPVTVSWNSGALTSGVHTFPAVLQSSGLYSLSSVVTVPSSSLGTQTYICNVNHKPSNTKVDKKVEPKSCDKTHTCPPCPAPELLGGPSVFLFPPKPKDTLMISRTPEVTCVVVDVSHEDPEVKFNWYVDGVEVHNAKTKPREEQYNSTYRVVSVLTVLHQDWLNGKEYKCKVSNKALPAPIEKTISKAKGQPREPQVYTLPPSREEMTKNQVSLTCLVKGFYPSDIAVEWESNGQPENNYKTTPPVLDSDGSFFLYSKLTVDKSRWQQGNVFSCSVMHEALHNHYTQKSLSLSPGK

SEQ ID NO: 147 - protein, 447 aa, Artificial Sequence
  PR001363 HC
QVQLVESGGGVVQPGRSLRLSCAASGFSFSSYAMHWVRQAPGRGLEWVAVIWYDGGDEDSIDSVKGRFTISRDDSKNTLYLQMNSLRAEDTAVYYCAREQARSFDLWGRGTLVTVSSASTKGPSVFPLAPSSKSTSGGTAALGCLVKDYFPEPVTVSWNSGALTSGVHTFPAVLQSSGLYSLSSVVTVPSSSLGTQTYICNVNHKPSNTKVDKKVEPKSCDKTHTCPPCPAPELLGGPSVFLFPPKPKDTLMISRTPEVTCVVVDVSHEDPEVKFNWYVDGVEVHNAKTKPREEQYNSTYRVVSVLTVLHQDWLNGKEYKCKVSNKALPAPIEKTISKAKGQPREPQVYTLPPSREEMTKNQVSLTCLVKGFYPSDIAVEWESNGQPENNYKTTPPVLDSDGSFFLYSKLTVDKSRWQQGNVFSCSVMHEALHNHYTQKSLSLSPGK

SEQ ID NO: 148 - protein, 447 aa, Artificial Sequence
  PR001364 HC, PR002572 HC, PR002573 HC
EVQLLESGGGVVQPGRSLRLSCAASGFTFSSFGMHWVRQAPGKGLEWVAVIWYDGSDKDYADSVKGRFTISRDTSKNTLYLQMNSLRAEDTAVYYCAREQARSFDLWGRGTLVTVSSASTKGPSVFPLAPSSKSTSGGTAALGCLVKDYFPEPVTVSWNSGALTSGVHTFPAVLQSSGLYSLSSVVTVPSSSLGTQTYICNVNHKPSNTKVDKKVEPKSCDKTHTCPPCPAPELLGGPSVFLFPPKPKDTLMISRTPEVTCVVVDVSHEDPEVKFNWYVDGVEVHNAKTKPREEQYNSTYRVVSVLTVLHQDWLNGKEYKCKVSNKALPAPIEKTISKAKGQPREPQVYTLPPSREEMTKNQVSLTCLVKGFYPSDIAVEWESNGQPENNYKTTPPVLDSDGSFFLYSKLTVDKSRWQQGNVFSCSVMHEALHNHYTQKSLSLSPGK

SEQ ID NO: 149 - protein, 447 aa, Artificial Sequence
  PR001365 HC
QVQLVQSGGGVVQPGRSLRLSCAASGFTFSSYGMHWVRQAPGKGLEWVAVIWYDGSDKDYADSVKGRFTISRDTSKNTLYLQMNSLRAEDTAVYYCAREQARSFDLWGRGTLVTVSSASTKGPSVFPLAPSSKSTSGGTAALGCLVKDYFPEPVTVSWNSGALTSGVHTFPAVLQSSGLYSLSSVVTVPSSSLGTQTYICNVNHKPSNTKVDKKVEPKSCDKTHTCPPCPAPELLGGPSVFLFPPKPKDTLMISRTPEVTCVVVDVSHEDPEVKFNWYVDGVEVHNAKTKPREEQYNSTYRVVSVLTVLHQDWLNGKEYKCKVSNKALPAPIEKTISKAKGQPREPQVYTLPPSREEMTKNQVSLTCLVKGFYPSDIAVEWESNGQPENNYKTTPPVLDSDGSFFLYSKLTVDKSRWQQGNVFSCSVMHEALHNHYTQKSLSLSPGK

SEQ ID NO: 150 - protein, 447 aa, Artificial Sequence
  PR001366 HC
QVQLVESGGGVVQPGRSLRLSCTASGFTFSSYGMHWVRQAPGKGLEWVAVKWYDGISQNFADSVKGRFTISRDNSKNTLYLQMNSLRAEDTAVYYCARDLARSFDIWGRGTLVTVSSASTKGPSVFPLAPSSKSTSGGTAALGCLVKDYFPEPVTVSWNSGALTSGVHTFPAVLQSSGLYSLSSVVTVPSSSLGTQTYICNVNHKPSNTKVDKKVEPKSCDKTHTCPPCPAPELLGGPSVFLFPPKPKDTLMISRTPEVTCVVVDVSHEDPEVKFNWYVDGVEVHNAKTKPREEQYNSTYRVVSVLTVLHQDWLNGKEYKCKVSNKALPAPIEKTISKAKGQPREPQVYTLPPSREEMTKNQVSLTCLVKGFYPSDIAVEWESNGQPENNYKTTPPVLDSDGSFFLYSKLTVDKSRWQQGNVFSCSVMHEALHNHYTQKSLSLSPGK

SEQ ID NO: 151 - protein, 447 aa, Artificial Sequence
  PR001367 HC, PR001417 HC
QVQLVESGGGVVQPGRSLRLSCAASGFSFSSYAMHWVRQAPGRGLEWVAVIWYDGGDEDYIDSVKGRFTISRDDSKNTLYLQMNSLRAEDTAVYYCAREQARSFDLWGRGTLVTVSSASTKGPSVFPLAPSSKSTSGGTAALGCLVKDYFPEPVTVSWNSGALTSGVHTFPAVLQSSGLYSLSSVVTVPSSSLGTQTYICNVNHKPSNTKVDKKVEPKSCDKTHTCPPCPAPELLGGPSVFLFPPKPKDTLMISRTPEVTCVVVDVSHEDPEVKFNWYVDGVEVHNAKTKPREEQYNSTYRVVSVLTVLHQDWLNGKEYKCKVSNKALPAPIEKTISKAKGQPREPQVYTLPPSREEMTKNQVSLTCLVKGFYPSDIAVEWESNGQPENNYKTTPPVLDSDGSFFLYSKLTVDKSRWQQGNVFSCSVMHEALHNHYTQKSLSLSPGK

SEQ ID NO: 152 - protein, 447 aa, Artificial Sequence
  PR001368 HC
QVQLVESGGGVVQPGRSLRLSCAASGFTFSTYGMHWVRQAPGKGLEWVAVIWYDGSDTDYADSVKGRFTISRDTSKNTLYLQMNSLRAEDTAVYYCAREQARSFDLWGRGTLVTVSSASTKGPSVFPLAPSSKSTSGGTAALGCLVKDYFPEPVTVSWNSGALTSGVHTFPAVLQSSGLYSLSSVVTVPSSSLGTQTYICNVNHKPSNTKVDKKVEPKSCDKTHTCPPCPAPELLGGPSVFLFPPKPKDTLMISRTPEVTCVVVDVSHEDPEVKFNWYVDGVEVHNAKTKPREEQYNSTYRVVSVLTVLHQDWLNGKEYKCKVSNKALPAPIEKTISKAKGQPREPQVYTLPPSREEMTKNQVSLTCLVKGFYPSDIAVEWESNGQPENNYKTTPPVLDSDGSFFLYSKLTVDKSRWQQGNVFSCSVMHEALHNHYTQKSLSLSPGK

SEQ ID NO: 153 - protein, 447 aa, Artificial Sequence
  PR001369 HC, PR002580 HC, PR002581 HC
QVQLVESGGGVVQPGRSLRLSCAASGFTFSNYGIHWVRQAPGKGLEWVAIMWYDGSNTDYADSVKGRFTISRDTSKNTLFLQMNSLRAEDTAVYYCAREQARSFDLWGRGTLVTVSSASTKGPSVFPLAPSSKSTSGGTAALGCLVKDYFPEPVTVSWNSGALTSGVHTFPAVLQSSGLYSLSSVVTVPSSSLGTQTYICNVNHKPSNTKVDKKVEPKSCDKTHTCPPCPAPELLGGPSVFLFPPKPKDTLMISRTPEVTCVVVDVSHEDPEVKFNWYVDGVEVHNAKTKPREEQYNSTYRVVSVLTVLHQDWLNGKEYKCKVSNKALPAPIEKTISKAKGQPREPQVYTLPPSREEMTKNQVSLTCLVKGFYPSDIAVEWESNGQPENNYKTTPPVLDSDGSFFLYSKLTVDKSRWQQGNVFSCSVMHEALHNHYTQKSLSLSPGK

SEQ ID NO: 154 - protein, 447 aa, Artificial Sequence
  PR001371 HC
QVQLVESGGGVVQPGRSLRLSCAASGFTFSSYGMLWVRQAPGKGLEWVAVAWYDGVSEDYADSVKGRFTISRDNSMNTLSLQMNSLRAEDTAVYYCAREQARSFDLWGRGTLVTVSSASTKGPSVFPLAPSSKSTSGGTAALGCLVKDYFPEPVTVSWNSGALTSGVHTFPAVLQSSGLYSLSSVVTVPSSSLGTQTYICNVNHKPSNTKVDKKVEPKSCDKTHTCPPCPAPELLGGPSVFLFPPKPKDTLMISRTPEVTCVVVDVSHEDPEVKFNWYVDGVEVHNAKTKPREEQYNSTYRVVSVLTVLHQDWLNGKEYKCKVSNKALPAPIEKTISKAKGQPREPQVYTLPPSREEMTKNQVSLTCLVKGFYPSDIAVEWESNGQPENNYKTTPPVLDSDGSFFLYSKLTVDKSRWQQGNVFSCSVMHEALHNHYTQKSLSLSPGK

SEQ ID NO: 155 - protein, 447 aa, Artificial Sequence
  PR001415 HC
EVQLVESGGGVVQPGRSLRLSCAASGFTFSNSGMHWVRQAPGKGLEWVAIMWYDGSNKDYADSVKGRFTISRDTSKNTLYLQMNSLRAEDTAVYYCAREQARSFDLWGRGTLVTVSSASTKGPSVFPLAPSSKSTSGGTAALGCLVKDYFPEPVTVSWNSGALTSGVHTFPAVLQSSGLYSLSSVVTVPSSSLGTQTYICNVNHKPSNTKVDKKVEPKSCDKTHTCPPCPAPELLGGPSVFLFPPKPKDTLMISRTPEVTCVVVDVSHEDPEVKFNWYVDGVEVHNAKTKPREEQYNSTYRVVSVLTVLHQDWLNGKEYKCKVSNKALPAPIEKTISKAKGQPREPQVYTLPPSREEMTKNQVSLTCLVKGFYPSDIAVEWESNGQPENNYKTTPPVLDSDGSFFLYSKLTVDKSRWQQGNVFSCSVMHEALHNHYTQKSLSLSPGK

SEQ ID NO: 156 - protein, 447 aa, Artificial Sequence
  PR001416 HC
QVQLVESGGGVVQPGRSLRLSCAASGFTFSTYGMHWVRQAPGKGLEWVAVIWYDGSDKDYADSVKGRFTISRDTSKNTLYLQMNSLRAEDTAVYYCAREQARSFDLWGRGTLVTVSSASTKGPSVFPLAPSSKSTSGGTAALGCLVKDYFPEPVTVSWNSGALTSGVHTFPAVLQSSGLYSLSSVVTVPSSSLGTQTYICNVNHKPSNTKVDKKVEPKSCDKTHTCPPCPAPELLGGPSVFLFPPKPKDTLMISRTPEVTCVVVDVSHEDPEVKFNWYVDGVEVHNAKTKPREEQYNSTYRVVSVLTVLHQDWLNGKEYKCKVSNKALPAPIEKTISKAKGQPREPQVYTLPPSREEMTKNQVSLTCLVKGFYPSDIAVEWESNGQPENNYKTTPPVLDSDGSFFLYSKLTVDKSRWQQGNVFSCSVMHEALHNHYTQKSLSLSPGK

SEQ ID NO: 157 - protein, 447 aa, Artificial Sequence
  PR001418 HC
QVQLVESGGGVVQPGRSLRLSCAASGFTFSSYGMHWVRQAPGKGLEWVAVIWYDGSDKDYADSVKGRFTISRDTSKNTLYLQMNSLRAEDTAVYYCAREQARSFDLWGRGTLVTVSSASTKGPSVFPLAPSSKSTSGGTAALGCLVKDYFPEPVTVSWNSGALTSGVHTFPAVLQSSGLYSLSSVVTVPSSSLGTQTYICNVNHKPSNTKVDKKVEPKSCDKTHTCPPCPAPELLGGPSVFLFPPKPKDTLMISRTPEVTCVVVDVSHEDPEVKFNWYVDGVEVHNAKTKPREEQYNSTYRVVSVLTVLHQDWLNGKEYKCKVSNKALPAPIEKTISKAKGQPREPQVYTLPPSREEMTKNQVSLTCLVKGFYPSDIAVEWESNGQPENNYKTTPPVLDSDGSFFLYSKLTVDKSRWQQGNVFSCSVMHEALHNHYTQKSLSLSPGK

SEQ ID NO: 158 - protein, 447 aa, Artificial Sequence
  PR001419 HC
QVQLVESGGGVVQPGRSLRLSCAASGFTFSSYGMHWVRQAPGKGLEWVAIIWYDGISKNYADSVKGRFTISRDMSNNTVYLQMNSLRAEDTAVYYCAKEQARSFDLWGRGTLVTVSSASTKGPSVFPLAPSSKSTSGGTAALGCLVKDYFPEPVTVSWNSGALTSGVHTFPAVLQSSGLYSLSSVVTVPSSSLGTQTYICNVNHKPSNTKVDKKVEPKSCDKTHTCPPCPAPELLGGPSVFLFPPKPKDTLMISRTPEVTCVVVDVSHEDPEVKFNWYVDGVEVHNAKTKPREEQYNSTYRVVSVLTVLHQDWLNGKEYKCKVSNKALPAPIEKTISKAKGQPREPQVYTLPPSREEMTKNQVSLTCLVKGFYPSDIAVEWESNGQPENNYKTTPPVLDSDGSFFLYSKLTVDKSRWQQGNVFSCSVMHEALHNHYTQKSLSLSPGK

SEQ ID NO: 159 - protein, 217 aa, Artificial Sequence
  PR000374 LC
DIQMTQSPSSLSASVGDRVTINCQASQSIDSNLAWFQQKPGQPPKLLIYRASNLASGVPDRFSGSGSGTDFTLTISSLEAEDVATYYCLGGVGAVSYRTSFGGGTKVEIKRTVAAPSVFIFPPSDEQLKSGTASVVCLLNNFYPREAKVQWKVDNALQSGNSQESVTEQDSKDSTYSLSSTLTLSKADYEKHKVYACEVTHQGLSSPVTKSFNRGEC

SEQ ID NO: 160 - protein, 216 aa, Artificial Sequence
  PR001352 LC, PR001371 LC
DIQLTQSPSSLSASVGDRVTITCRASQTINNWLAWYQQKPGKAPKLLIYKASSLESGVPSRFSGSGSGTEFTLTISSLQPDDFATYYCQQYNSYSPMYTFGQGTKVEIKRTVAAPSVFIFPPSDEQLKSGTASVVCLLNNFYPREAKVQWKVDNALQSGNSQESVTEQDSKDSTYSLSSTLTLSKADYEKHKVYACEVTHQGLSSPVTKSFNRGEC

SEQ ID NO: 161 - protein, 216 aa, Artificial Sequence
  PR001353 LC
DIVMTQSPSTLSASVGDRVTITCRASQSISSWLAWYQQKPGKAPKLLIYKASSLESGVPSRFSGSGSGTEFTLTISSLQPDDFATYYCQQYKSYSPMYTFGQGTKVEIKRTVAAPSVFIFPPSDEQLKSGTASVVCLLNNFYPREAKVQWKVDNALQSGNSQESVTEQDSKDSTYSLSSTLTLSKADYEKHKVYACEVTHQGLSSPVTKSFNRGEC

SEQ ID NO: 162 - protein, 216 aa, Artificial Sequence
  PR001354 LC, PR002564 LC, PR002567 LC
DIVMTQSPSSLSASVGDRVTITCRASQTINNWLAWYQQKPGKAPKLLIYKASSLESGVPSRFSGSGSGTEFTLTISSLQPDDFATYYCQQYNSYSPMYTFGQGTKVEIKRTVAAPSVFIFPPSDEQLKSGTASVVCLLNNFYPREAKVQWKVDNALQSGNSQESVTEQDSKDSTYSLSSTLTLSKADYEKHKVYACEVTHQGLSSPVTKSFNRGEC

SEQ ID NO: 163 - protein, 216 aa, Artificial Sequence
  PR001355 LC
DIQMTQSPSSLSASVGDRVTITCRASQTMNNWLAWYQQKPGKAPKLLIYKASSLESGVPSRFSGSGSGTEFTLTISSLQPDDSATYYCQQYNSYSPMYTFGQGTKLEIKRTVAAPSVFIFPPSDEQLKSGTASVVCLLNNFYPREAKVQWKVDNALQSGNSQESVTEQDSKDSTYSLSSTLTLSKADYEKHKVYACEVTHQGLSSPVTKSFNRGEC

SEQ ID NO: 164 - protein, 216 aa, Artificial Sequence
  PR001356 LC, PR002570 LC, PR002571 LC
DIVMTQSPSTLSASVGDRVTITCRASQSINNWLAWYQQKPGKAPKLLIYKASSLESGVPSRFSGSGSGTEFTLTISSLQPDDFATYYCQQYKSYSPMYTFGQGTKVEIKRTVAAPSVFIFPPSDEQLKSGTASVVCLLNNFYPREAKVQWKVDNALQSGNSQESVTEQDSKDSTYSLSSTLTLSKADYEKHKVYACEVTHQGLSSPVTKSFNRGEC

SEQ ID NO: 165 - protein, 216 aa, Artificial Sequence
  PR001357 LC
DIQLTQSPYSLSASVGDRVTITCRASQTINNWLAWYQQKPGKAPKLLIYKASSLESGVPSRFSGSGSGTEFTLTISSLQPDDFATYYCQQYKLYSPMYTFGQGTKVEIKRTVAAPSVFIFPPSDEQLKSGTASVVCLLNNFYPREAKVQWKVDNALQSGNSQESVTEQDSKDSTYSLSSTLTLSKADYEKHKVYACEVTHQGLSSPVTKSFNRGEC

SEQ ID NO: 166 - protein, 216 aa, Artificial Sequence
  PR001358 LC
DIVMTQSPSTLSASVGDRVTITCRASQSINSWLAWYQQKPGKAPKLLIYKASNLESGVPSRFSGSGSGTEFTLTISSLQPDDFATYYCQQYKSYSPMYTFGQGTKVDIKRTVAAPSVFIFPPSDEQLKSGTASVVCLLNNFYPREAKVQWKVDNALQSGNSQESVTEQDSKDSTYSLSSTLTLSKADYEKHKVYACEVTHQGLSSPVTKSFNRGEC

SEQ ID NO: 167 - protein, 216 aa, Artificial Sequence
  PR001359 LC
DIVMTQSPSTLSASVGDRVTITCRASQSVNNWLAWYQQKPGKAPKLLIYKASSLESGVPSRFSGSGSGTEFTLTISSLQPDDFATYYCQQYKSYSPMYTFGQGTKVEIKRTVAAPSVFIFPPSDEQLKSGTASVVCLLNNFYPREAKVQWKVDNALQSGNSQESVTEQDSKDSTYSLSSTLTLSKADYEKHKVYACEVTHQGLSSPVTKSFNRGEC

SEQ ID NO: 168 - protein, 216 aa, Artificial Sequence
  PR001360 LC
DIQMTQSPSTLSASVGDRVTITCRASQTINNWLAWYQQKPGKAPKLLIYKASSLESGVPSRFSGSGSGTEFTLTISSLQPDDFATYYCQQYNIYSPMYTFGQGTKVEIKRTVAAPSVFIFPPSDEQLKSGTASVVCLLNNFYPREAKVQWKVDNALQSGNSQESVTEQDSKDSTYSLSSTLTLSKADYEKHKVYACEVTHQGLSSPVTKSFNRGEC

SEQ ID NO: 169 - protein, 216 aa, Artificial Sequence
  PR001361 LC, PR001366 LC
DIQLTQSPSTLSASVGDRVTITCRASQSINSWLAWYQQKPGKAPKLLIYKASSLESGVPSRFSGSGSGTEFTLTISSLQPDDFATYYCQQYKSYSPMYTFGQGTKVDIKRTVAAPSVFIFPPSDEQLKSGTASVVCLLNNFYPREAKVQWKVDNALQSGNSQESVTEQDSKDSTYSLSSTLTLSKADYEKHKVYACEVTHQGLSSPVTKSFNRGEC

SEQ ID NO: 170 - protein, 216 aa, Artificial Sequence
  PR001362 LC, PR001368 LC
DIVMTQSPSTLSASVGDRVTITCRASQSINSWLAWYQQKPGKAPKLLIYKASSLESGVPSRFSGSGSGTEFTLTISSLQPDDFATYYCQQYKSYSPMYTFGQGTKVEIKRTVAAPSVFIFPPSDEQLKSGTASVVCLLNNFYPREAKVQWKVDNALQSGNSQESVTEQDSKDSTYSLSSTLTLSKADYEKHKVYACEVTHQGLSSPVTKSFNRGEC

SEQ ID NO: 171 - protein, 216 aa, Artificial Sequence
  PR001363 LC, PR001367 LC
DVVMTQSPSTLSASVGDRVTITCRASQTINNWLAWYQQKPGKAPKLLIYKASSLESGVPSRFSGSGSGTEFTLTISSLQPDDFATYYCQQYNSYSPMYTFGQGTKVEIKRTVAAPSVFIFPPSDEQLKSGTASVVCLLNNFYPREAKVQWKVDNALQSGNSQESVTEQDSKDSTYSLSSTLTLSKADYEKHKVYACEVTHQGLSSPVTKSFNRGEC

SEQ ID NO: 172 - protein, 216 aa, Artificial Sequence
  PR001364 LC, PR001369 LC, PR001415 LC, PR001416 LC, PR002574 LC, PR002577 LC, PR002582 LC, PR002585 LC
DIVMTQSPSTLSASVGDRVTITCRASQTINNWLAWYQQKPGKAPKLLIYKASSLESGVPSRFSGSGSGTEFTLTISSLQPDDFATYYCQQYNSYSPMYTFGQGTKVEIKRTVAAPSVFIFPPSDEQLKSGTASVVCLLNNFYPREAKVQWKVDNALQSGNSQESVTEQDSKDSTYSLSSTLTLSKADYEKHKVYACEVTHQGLSSPVTKSFNRGEC

SEQ ID NO: 173 - protein, 216 aa, Artificial Sequence
  PR001365 LC
DIQMTQSPYSLSASVGDRVTITCRASQTINNWLAWYQQKPGKAPKLLIYKASSLESGVPSRFSGSGSGTEFTLTISSLQPDDFATYYCQQYKLYSPMYTFGQGTKVEIKRTVAAPSVFIFPPSDEQLKSGTASVVCLLNNFYPREAKVQWKVDNALQSGNSQESVTEQDSKDSTYSLSSTLTLSKADYEKHKVYACEVTHQGLSSPVTKSFNRGEC

SEQ ID NO: 174 - protein, 216 aa, Artificial Sequence
  PR001370 LC
DIVMTQSPSTLSASVGDRVTITCRASQSINNWLAWYQQKPGKAPKLLIYKASSLESGVPSRFSGSGSGTEFTLTISSLQPDDFATYYCQQYNSYSPMYTFGQGTKVDIKRTVAAPSVFIFPPSDEQLKSGTASVVCLLNNFYPREAKVQWKVDNALQSGNSQESVTEQDSKDSTYSLSSTLTLSKADYEKHKVYACEVTHQGLSSPVTKSFNRGEC

SEQ ID NO: 175 - protein, 216 aa, Artificial Sequence
  PR001417 LC
DVVMTQSPSTLSASVGDRVTITCRASQSINSWLAWYQQKPGKAPKLLIYKASSLESGVPSRFSGSGSGTEFTLTISSLQPDDFATYYCQQYNSYSPMYTFGQGTKVEIKRTVAAPSVFIFPPSDEQLKSGTASVVCLLNNFYPREAKVQWKVDNALQSGNSQESVTEQDSKDSTYSLSSTLTLSKADYEKHKVYACEVTHQGLSSPVTKSFNRGEC

SEQ ID NO: 176 - protein, 216 aa, Artificial Sequence
  PR001418 LC
DIVMTQSPSTLSASVGDRVTITCRASQTINNWLAWYQQKPGKAPKLLIYKASSLESGVPSRFSGSGSGTEFTLTISSLQPDDFATYYCQQYNSYSPMYTFGQGTKLEIKRTVAAPSVFIFPPSDEQLKSGTASVVCLLNNFYPREAKVQWKVDNALQSGNSQESVTEQDSKDSTYSLSSTLTLSKADYEKHKVYACEVTHQGLSSPVTKSFNRGEC

SEQ ID NO: 177 - protein, 216 aa, Artificial Sequence
  PR001419 LC
DIQLTQSPSTLSASVGDRVTITCRASQSISSWLAWYQQKPGKAPKLLIYKASSLESGVPSRFSGSGSGTEFTLTISSLQPDDFATYYCQQYNSYSPMYTFGQGTKVEIKRTVAAPSVFIFPPSDEQLKSGTASVVCLLNNFYPREAKVQWKVDNALQSGNSQESVTEQDSKDSTYSLSSTLTLSKADYEKHKVYACEVTHQGLSSPVTKSFNRGEC

SEQ ID NO: 178 - protein, 6 aa, Artificial Sequence
  PR002564 HCDR2 Chothia, PR002565 HCDR2 Chothia, PR002566 HCDR2 Chothia, PR002574 HCDR2 Chothia, PR002575 HCDR2 Chothia, PR002576 HCDR2 Chothia
WYEGSD

SEQ ID NO: 179 - protein, 6 aa, Artificial Sequence
  PR002567 HCDR2 Chothia, PR002568 HCDR2 Chothia, PR002569 HCDR2 Chothia, PR002577 HCDR2 Chothia, PR002578 HCDR2 Chothia, PR002579 HCDR2 Chothia
WYDASD

SEQ ID NO: 180 - protein, 6 aa, Artificial Sequence
  PR002570 HCDR2 Chothia
WYEGVS

SEQ ID NO: 181 - protein, 6 aa, Artificial Sequence
  PR002571 HCDR2 Chothia
WYDAVS

SEQ ID NO: 182 - protein, 6 aa, Artificial Sequence
  PR002582 HCDR2 Chothia, PR002583 HCDR2 Chothia, PR002584 HCDR2 Chothia
WYEGSN

SEQ ID NO: 183 - protein, 6 aa, Artificial Sequence
  PR002585 HCDR2 Chothia, PR002586 HCDR2 Chothia, PR002587 HCDR2 Chothia
WYDASN

SEQ ID NO: 184 - protein, 11 aa, Artificial Sequence
  PR002562 LCDR3 Chothia, PR002565 LCDR3 Chothia, PR002568 LCDR3 Chothia, PR002572 LCDR3 Chothia, PR002575 LCDR3 Chothia, PR002578 LCDR3 Chothia, PR002580 LCDR3 Chothia, PR002583 LCDR3 Chothia, PR002586
QQYQSYSPMYT

SEQ ID NO: 185 - protein, 11 aa, Artificial Sequence
  PR002563 LCDR3 Chothia, PR002566 LCDR3 Chothia, PR002569 LCDR3 Chothia, PR002573 LCDR3 Chothia, PR002576 LCDR3 Chothia, PR002579 LCDR3 Chothia, PR002581 LCDR3 Chothia, PR002584 LCDR3 Chothia, PR002587
QQYNAYSPMYT

SEQ ID NO: 186 - protein, 117 aa, Artificial Sequence
  PR002564 VH, PR002565 VH, PR002566 VH
QVQLVQSGGGVVQPGRSLRLSCAASGFTFSSYGMHWVRQAPGKGLEWVAIMWYEGSDKDYADSVKGRFTISRDTSKNTLYLQMNSLRAEDTAVYYCAREQARSFDLWGRGTLVTVSS

SEQ ID NO: 187 - protein, 117 aa, Artificial Sequence
  PR002567 VH, PR002568 VH, PR002569 VH
QVQLVQSGGGVVQPGRSLRLSCAASGFTFSSYGMHWVRQAPGKGLEWVAIMWYDASDKDYADSVKGRFTISRDTSKNTLYLQMNSLRAEDTAVYYCAREQARSFDLWGRGTLVTVSS

SEQ ID NO: 188 - protein, 117 aa, Artificial Sequence
  PR002570 VH
QVQLVESGGGVVQPGRSLRLSCAASGFTFSSYGMHWVRQAPGKGLEWVAVAWYEGVSEDYADSVKGRFTISRDNAKNTLYLQMNSLRAEDTAVYYCAREQARSFDLWGRGTLVTVSS

SEQ ID NO: 189 - protein, 117 aa, Artificial Sequence
  PR002571 VH
QVQLVESGGGVVQPGRSLRLSCAASGFTFSSYGMHWVRQAPGKGLEWVAVAWYDAVSEDYADSVKGRFTISRDNAKNTLYLQMNSLRAEDTAVYYCAREQARSFDLWGRGTLVTVSS

SEQ ID NO: 190 - protein, 117 aa, Artificial Sequence
  PR002574 VH, PR002575 VH, PR002576 VH
EVQLLESGGGVVQPGRSLRLSCAASGFTFSSFGMHWVRQAPGKGLEWVAVIWYEGSDKDYADSVKGRFTISRDTSKNTLYLQMNSLRAEDTAVYYCAREQARSFDLWGRGTLVTVSS

SEQ ID NO: 191 - protein, 117 aa, Artificial Sequence
  PR002577 VH, PR002578 VH, PR002579 VH
EVQLLESGGGVVQPGRSLRLSCAASGFTFSSFGMHWVRQAPGKGLEWVAVIWYDASDKDYADSVKGRFTISRDTSKNTLYLQMNSLRAEDTAVYYCAREQARSFDLWGRGTLVTVSS

SEQ ID NO: 192 - protein, 117 aa, Artificial Sequence
  PR002582 VH, PR002583 VH, PR002584 VH
QVQLVESGGGVVQPGRSLRLSCAASGFTFSNYGIHWVRQAPGKGLEWVAIMWYEGSNTDYADSVKGRFTISRDTSKNTLFLQMNSLRAEDTAVYYCAREQARSFDLWGRGTLVTVSS

SEQ ID NO: 193 - protein, 117 aa, Artificial Sequence
  PR002585 VH, PR002586 VH, PR002587 VH
QVQLVESGGGVVQPGRSLRLSCAASGFTFSNYGIHWVRQAPGKGLEWVAIMWYDASNTDYADSVKGRFTISRDTSKNTLFLQMNSLRAEDTAVYYCAREQARSFDLWGRGTLVTVSS

SEQ ID NO: 194 - protein, 109 aa, Artificial Sequence
  PR002562 VL, PR002565 VL, PR002568 VL
DIVMTQSPSSLSASVGDRVTITCRASQTINNWLAWYQQKPGKAPKLLIYKASSLESGVPSRFSGSGSGTEFTLTISSLQPDDFATYYCQQYQSYSPMYTFGQGTKVEIK

SEQ ID NO: 195 - protein, 109 aa, Artificial Sequence
  PR002563 VL, PR002566 VL, PR002569 VL
DIVMTQSPSSLSASVGDRVTITCRASQTINNWLAWYQQKPGKAPKLLIYKASSLESGVPSRFSGSGSGTEFTLTISSLQPDDFATYYCQQYNAYSPMYTFGQGTKVEIK

SEQ ID NO: 196 - protein, 109 aa, Artificial Sequence
  PR002572 VL, PR002575 VL, PR002578 VL, PR002580 VL, PR002583 VL, PR002586 VL
DIVMTQSPSTLSASVGDRVTITCRASQTINNWLAWYQQKPGKAPKLLIYKASSLESGVPSRFSGSGSGTEFTLTISSLQPDDFATYYCQQYQSYSPMYTFGQGTKVEIK

SEQ ID NO: 197 - protein, 109 aa, Artificial Sequence
  PR002573 VL, PR002576 VL, PR002579 VL, PR002581 VL, PR002584 VL, PR002587 VL
DIVMTQSPSTLSASVGDRVTITCRASQTINNWLAWYQQKPGKAPKLLIYKASSLESGVPSRFSGSGSGTEFTLTISSLQPDDFATYYCQQYNAYSPMYTFGQGTKVEIK

SEQ ID NO: 198 - protein, 447 aa, Artificial Sequence
  PR002564 HC, PR002565 HC, PR002566 HC
QVQLVQSGGGVVQPGRSLRLSCAASGFTFSSYGMHWVRQAPGKGLEWVAIMWYEGSDKDYADSVKGRFTISRDTSKNTLYLQMNSLRAEDTAVYYCAREQARSFDLWGRGTLVTVSSASTKGPSVFPLAPSSKSTSGGTAALGCLVKDYFPEPVTVSWNSGALTSGVHTFPAVLQSSGLYSLSSVVTVPSSSLGTQTYICNVNHKPSNTKVDKKVEPKSCDKTHTCPPCPAPELLGGPSVFLFPPKPKDTLMISRTPEVTCVVVDVSHEDPEVKFNWYVDGVEVHNAKTKPREEQYNSTYRVVSVLTVLHQDWLNGKEYKCKVSNKALPAPIEKTISKAKGQPREPQVYTLPPSREEMTKNQVSLTCLVKGFYPSDIAVEWESNGQPENNYKTTPPVLDSDGSFFLYSKLTVDKSRWQQGNVFSCSVMHEALHNHYTQKSLSLSPGK

SEQ ID NO: 199 - protein, 447 aa, Artificial Sequence
  PR002567 HC, PR002568 HC, PR002569 HC
QVQLVQSGGGVVQPGRSLRLSCAASGFTFSSYGMHWVRQAPGKGLEWVAIMWYDASDKDYADSVKGRFTISRDTSKNTLYLQMNSLRAEDTAVYYCAREQARSFDLWGRGTLVTVSSASTKGPSVFPLAPSSKSTSGGTAALGCLVKDYFPEPVTVSWNSGALTSGVHTFPAVLQSSGLYSLSSVVTVPSSSLGTQTYICNVNHKPSNTKVDKKVEPKSCDKTHTCPPCPAPELLGGPSVFLFPPKPKDTLMISRTPEVTCVVVDVSHEDPEVKFNWYVDGVEVHNAKTKPREEQYNSTYRVVSVLTVLHQDWLNGKEYKCKVSNKALPAPIEKTISKAKGQPREPQVYTLPPSREEMTKNQVSLTCLVKGFYPSDIAVEWESNGQPENNYKTTPPVLDSDGSFFLYSKLTVDKSRWQQGNVFSCSVMHEALHNHYTQKSLSLSPGK

SEQ ID NO: 200 - protein, 447 aa, Artificial Sequence
  PR002570 HC
QVQLVESGGGVVQPGRSLRLSCAASGFTFSSYGMHWVRQAPGKGLEWVAVAWYEGVSEDYADSVKGRFTISRDNAKNTLYLQMNSLRAEDTAVYYCAREQARSFDLWGRGTLVTVSSASTKGPSVFPLAPSSKSTSGGTAALGCLVKDYFPEPVTVSWNSGALTSGVHTFPAVLQSSGLYSLSSVVTVPSSSLGTQTYICNVNHKPSNTKVDKKVEPKSCDKTHTCPPCPAPELLGGPSVFLFPPKPKDTLMISRTPEVTCVVVDVSHEDPEVKFNWYVDGVEVHNAKTKPREEQYNSTYRVVSVLTVLHQDWLNGKEYKCKVSNKALPAPIEKTISKAKGQPREPQVYTLPPSREEMTKNQVSLTCLVKGFYPSDIAVEWESNGQPENNYKTTPPVLDSDGSFFLYSKLTVDKSRWQQGNVFSCSVMHEALHNHYTQKSLSLSPGK

SEQ ID NO: 201 - protein, 447 aa, Artificial Sequence
  PR002571 HC
QVQLVESGGGVVQPGRSLRLSCAASGFTFSSYGMHWVRQAPGKGLEWVAVAWYDAVSEDYADSVKGRFTISRDNAKNTLYLQMNSLRAEDTAVYYCAREQARSFDLWGRGTLVTVSSASTKGPSVFPLAPSSKSTSGGTAALGCLVKDYFPEPVTVSWNSGALTSGVHTFPAVLQSSGLYSLSSVVTVPSSSLGTQTYICNVNHKPSNTKVDKKVEPKSCDKTHTCPPCPAPELLGGPSVFLFPPKPKDTLMISRTPEVTCVVVDVSHEDPEVKFNWYVDGVEVHNAKTKPREEQYNSTYRVVSVLTVLHQDWLNGKEYKCKVSNKALPAPIEKTISKAKGQPREPQVYTLPPSREEMTKNQVSLTCLVKGFYPSDIAVEWESNGQPENNYKTTPPVLDSDGSFFLYSKLTVDKSRWQQGNVFSCSVMHEALHNHYTQKSLSLSPGK

SEQ ID NO: 202 - protein, 447 aa, Artificial Sequence
  PR002574 HC, PR002575 HC, PR002576 HC
EVQLLESGGGVVQPGRSLRLSCAASGFTFSSFGMHWVRQAPGKGLEWVAVIWYEGSDKDYADSVKGRFTISRDTSKNTLYLQMNSLRAEDTAVYYCAREQARSFDLWGRGTLVTVSSASTKGPSVFPLAPSSKSTSGGTAALGCLVKDYFPEPVTVSWNSGALTSGVHTFPAVLQSSGLYSLSSVVTVPSSSLGTQTYICNVNHKPSNTKVDKKVEPKSCDKTHTCPPCPAPELLGGPSVFLFPPKPKDTLMISRTPEVTCVVVDVSHEDPEVKFNWYVDGVEVHNAKTKPREEQYNSTYRVVSVLTVLHQDWLNGKEYKCKVSNKALPAPIEKTISKAKGQPREPQVYTLPPSREEMTKNQVSLTCLVKGFYPSDIAVEWESNGQPENNYKTTPPVLDSDGSFFLYSKLTVDKSRWQQGNVFSCSVMHEALHNHYTQKSLSLSPGK

SEQ ID NO: 203 - protein, 447 aa, Artificial Sequence
  PR002577 HC, PR002578 HC, PR002579 HC
EVQLLESGGGVVQPGRSLRLSCAASGFTFSSFGMHWVRQAPGKGLEWVAVIWYDASDKDYADSVKGRFTISRDTSKNTLYLQMNSLRAEDTAVYYCAREQARSFDLWGRGTLVTVSSASTKGPSVFPLAPSSKSTSGGTAALGCLVKDYFPEPVTVSWNSGALTSGVHTFPAVLQSSGLYSLSSVVTVPSSSLGTQTYICNVNHKPSNTKVDKKVEPKSCDKTHTCPPCPAPELLGGPSVFLFPPKPKDTLMISRTPEVTCVVVDVSHEDPEVKFNWYVDGVEVHNAKTKPREEQYNSTYRVVSVLTVLHQDWLNGKEYKCKVSNKALPAPIEKTISKAKGQPREPQVYTLPPSREEMTKNQVSLTCLVKGFYPSDIAVEWESNGQPENNYKTTPPVLDSDGSFFLYSKLTVDKSRWQQGNVFSCSVMHEALHNHYTQKSLSLSPGK

SEQ ID NO: 204 - protein, 447 aa, Artificial Sequence
  PR002582 HC, PR002583 HC, PR002584 HC
QVQLVESGGGVVQPGRSLRLSCAASGFTFSNYGIHWVRQAPGKGLEWVAIMWYEGSNTDYADSVKGRFTISRDTSKNTLFLQMNSLRAEDTAVYYCAREQARSFDLWGRGTLVTVSSASTKGPSVFPLAPSSKSTSGGTAALGCLVKDYFPEPVTVSWNSGALTSGVHTFPAVLQSSGLYSLSSVVTVPSSSLGTQTYICNVNHKPSNTKVDKKVEPKSCDKTHTCPPCPAPELLGGPSVFLFPPKPKDTLMISRTPEVTCVVVDVSHEDPEVKFNWYVDGVEVHNAKTKPREEQYNSTYRVVSVLTVLHQDWLNGKEYKCKVSNKALPAPIEKTISKAKGQPREPQVYTLPPSREEMTKNQVSLTCLVKGFYPSDIAVEWESNGQPENNYKTTPPVLDSDGSFFLYSKLTVDKSRWQQGNVFSCSVMHEALHNHYTQKSLSLSPGK

SEQ ID NO: 205 - protein, 447 aa, Artificial Sequence
  PR002585 HC, PR002586 HC, PR002587 HC
QVQLVESGGGVVQPGRSLRLSCAASGFTFSNYGIHWVRQAPGKGLEWVAIMWYDASNTDYADSVKGRFTISRDTSKNTLFLQMNSLRAEDTAVYYCAREQARSFDLWGRGTLVTVSSASTKGPSVFPLAPSSKSTSGGTAALGCLVKDYFPEPVTVSWNSGALTSGVHTFPAVLQSSGLYSLSSVVTVPSSSLGTQTYICNVNHKPSNTKVDKKVEPKSCDKTHTCPPCPAPELLGGPSVFLFPPKPKDTLMISRTPEVTCVVVDVSHEDPEVKFNWYVDGVEVHNAKTKPREEQYNSTYRVVSVLTVLHQDWLNGKEYKCKVSNKALPAPIEKTISKAKGQPREPQVYTLPPSREEMTKNQVSLTCLVKGFYPSDIAVEWESNGQPENNYKTTPPVLDSDGSFFLYSKLTVDKSRWQQGNVFSCSVMHEALHNHYTQKSLSLSPGK

SEQ ID NO: 206 - protein, 216 aa, Artificial Sequence
  PR002562 LC, PR002565 LC, PR002568 LC
DIVMTQSPSSLSASVGDRVTITCRASQTINNWLAWYQQKPGKAPKLLIYKASSLESGVPSRFSGSGSGTEFTLTISSLQPDDFATYYCQQYQSYSPMYTFGQGTKVEIKRTVAAPSVFIFPPSDEQLKSGTASVVCLLNNFYPREAKVQWKVDNALQSGNSQESVTEQDSKDSTYSLSSTLTLSKADYEKHKVYACEVTHQGLSSPVTKSFNRGEC

SEQ ID NO: 207 - protein, 216 aa, Artificial Sequence
  PR002563 LC, PR002566 LC, PR002569 LC
DIVMTQSPSSLSASVGDRVTITCRASQTINNWLAWYQQKPGKAPKLLIYKASSLESGVPSRFSGSGSGTEFTLTISSLQPDDFATYYCQQYNAYSPMYTFGQGTKVEIKRTVAAPSVFIFPPSDEQLKSGTASVVCLLNNFYPREAKVQWKVDNALQSGNSQESVTEQDSKDSTYSLSSTLTLSKADYEKHKVYACEVTHQGLSSPVTKSFNRGEC

SEQ ID NO: 208 - protein, 216 aa, Artificial Sequence
  PR002572 LC, PR002575 LC, PR002578 LC, PR002580 LC, PR002583 LC, PR002586 LC
DIVMTQSPSTLSASVGDRVTITCRASQTINNWLAWYQQKPGKAPKLLIYKASSLESGVPSRFSGSGSGTEFTLTISSLQPDDFATYYCQQYQSYSPMYTFGQGTKVEIKRTVAAPSVFIFPPSDEQLKSGTASVVCLLNNFYPREAKVQWKVDNALQSGNSQESVTEQDSKDSTYSLSSTLTLSKADYEKHKVYACEVTHQGLSSPVTKSFNRGEC

SEQ ID NO: 209 - protein, 216 aa, Artificial Sequence
  PR002573 LC, PR002576 LC, PR002579 LC, PR002581 LC, PR002584 LC, PR002587 LC
DIVMTQSPSTLSASVGDRVTITCRASQTINNWLAWYQQKPGKAPKLLIYKASSLESGVPSRFSGSGSGTEFTLTISSLQPDDFATYYCQQYNAYSPMYTFGQGTKVEIKRTVAAPSVFIFPPSDEQLKSGTASVVCLLNNFYPREAKVQWKVDNALQSGNSQESVTEQDSKDSTYSLSSTLTLSKADYEKHKVYACEVTHQGLSSPVTKSFNRGEC